European Patent Specification EP 4 021 496 B1, published December 17, 2025. Title: COMPOSITIONS AND METHODS FOR DELIVERY OF NUCLEIC ACIDS TO CELLS. Applicant: YALE UNIVERSITY QUIJANO, ELIAS GLAZER, PETER. The sequence listing filed with the application follows.

SEQUENCE LISTING (93 sequences)

SEQ ID NO: 1 - protein, 116 aa, Artificial Sequence
  synthetic polypeptide
EVQLVESGGGLVKPGGSRKLSCAASGFTFSDYGMHWVRQAPEKGLEWVAYISSGSSTIYYADTVKGRFTISRDNAKNTLFLQMTSLRSEDTAMYYCARRGLLLDYWGQGTTLTVSS

SEQ ID NO: 2 - protein, 116 aa, Artificial Sequence
  synthetic polypeptide
EVQLVESGGGLVKPGGSRKLSCAASGFTFSNYGMHWVRQAPEKGLEWVAYISSGSSTIYYADTVKGRFTISRDNAKNTLFLQMTSLRSEDTAMYYCARRGLLLDYWGQGTTLTVSS

SEQ ID NO: 3 - protein, 116 aa, Artificial Sequence
  synthetic polypeptide
EVQLVQSGGGLIQPGGSLRLSCAASGFTFSNYGMHWVRQAPGKGLEWVSYISSGSSTIYYADSVKGRFTISRDNSKNTLYLQMNSLRAEDTAVYYCARRGLLLDYWGQGTTVTVSS

SEQ ID NO: 4 - protein, 116 aa, Artificial Sequence
  synthetic polypeptide
EVQLVESGGGLIQPGGSLRLSCAASGFTFSNYGMHWVRQAPGKGLEWVSYISSGSSTIYYADSVKGRFTISRDNSKNTLYLQMTSLRAEDTAVYYCARRGLLLDYWGQGTTLTVSS

SEQ ID NO: 5 - protein, 116 aa, Artificial Sequence
  synthetic polypeptide
EVQLQESGGGVVQPGGSLRLSCAASGFTFSNYGMHWIRQAPGKGLEWVSYISSGSSTIYYADSVKGRFTISRDNSKNTLYLQMNSLRSEDTAVYYCARRGLLLDYWGQGTLVTVSS

SEQ ID NO: 6 - protein, 116 aa, Artificial Sequence
  synthetic polypeptide
EVQLVESGGGLVQPGGSLRLSCSASGFTFSNYGMHWVRQAPGKGLEYVSYISSGSSTIYYADTVKGRFTISRDNSKNTLYLQMSSLRAEDTAVYYCVKRGLLLDYWGQGTLVTVSS

SEQ ID NO: 7 - protein, 111 aa, Artificial Sequence
  synthetic polypeptide
DIVLTQSPASLAVSLGQRATISCRASKSVSTSSYSYMHWYQQKPGQPPKLLIKYASYLESGVPARFSGSGSGTDFTLNIHPVEEEDAATYYCQHSREFPWTFGGGTKLEIK

SEQ ID NO: 8 - protein, 111 aa, Artificial Sequence
  synthetic polypeptide
DIVLTQSPASLAVSLGQRATISCRASKSVSTSSYSYMHWYQQKPGQPPKLLIKYASYLESGVPARFSGSGSGTDFHLNIHPVEEEDAATYYCQHSREFPWTFGGGTKLELK

SEQ ID NO: 9 - protein, 111 aa, Artificial Sequence
  synthetic polypeptide
DIQMTQSPSSLSASVGDRVTITCRASKSVSTSSYSYLAWYQQKPEKAPKLLIKYASYLQSGVPSRFSGSGSGTDFTLTISSLQPEDFATYYCQHSREFPWTFGAGTKLELK

SEQ ID NO: 10 - protein, 111 aa, Artificial Sequence
  synthetic polypeptide
DIQMTQSPSSLSASVGDRVTISCRASKSVSTSSYSYMHWYQQKPEKAPKLLIKYASYLQSGVPSRFSGSGSGTDFTLTISSLQPEDVATYYCQHSREFPWTFGAGTKLELK

SEQ ID NO: 11 - protein, 111 aa, Artificial Sequence
  synthetic polypeptide
DIVLTQSPASLAVSPGQRATITCRASKSVSTSSYSYMHWYQQKPGQPPKLLIYYASYLESGVPARFSGSGSGTDFTLTINPVEANDTANYYCQHSREFPWTFGQGTKVEIK

SEQ ID NO: 12 - protein, 465 aa, Artificial Sequence
  synthetic polypeptide
MGWSCIILFLVATATGVHSEVQLVESGGGLVKPGGSRKLSCAASGFTFSDYGMHWVRQAPEKGLEWVAYISSGSSTIYYADTVKGRFTISRDNAKNTLFLQMTSLRSEDTAMYYCARRGLLLDYWGQGTTLTVSAASTKGPSVFPLAPSSKSTSGGTAALGCLVKDYFPEPVTVSWNSGALTSGVHTFPAVLQSSGLYSLSSVVTVPSSSLGTQTYICNVNHKPSNTKVDKKVEPKSCDKTHTCPPCPAPELLGGPSVFLFPPKPKDTLMISRTPEVTCVVVDVSHEDPEVKFNWYVDGVEVHNAKTKPREEQYNSTYRVVSVLTVLHQDWLNGKEYKCKVSNKALPAPIEKTISKAKGQPREPQVYTLPPSRDELTKNQVSLTCLVKGFYPSDIAVEWESNGQPENNYKTTPPVLDSDGSFFLYSKLTVDKSRWQQGNVFSCSVMHEALHNHYTQKSLSLSPGK

SEQ ID NO: 13 - protein, 465 aa, Artificial Sequence
  synthetic polypeptide
MGWSCIILFLVATATGVHSEVQLVESGGGLVKPGGSRKLSCAASGFTFSNYGMHWVRQAPEKGLEWVAYISSGSSTIYYADTVKGRFTISRDNAKNTLFLQMTSLRSEDTAMYYCARRGLLLDYWGQGTTLTVSAASTKGPSVFPLAPSSKSTSGGTAALGCLVKDYFPEPVTVSWNSGALTSGVHTFPAVLQSSGLYSLSSVVTVPSSSLGTQTYICNVNHKPSNTKVDKKVEPKSCDKTHTCPPCPAPELLGGPSVFLFPPKPKDTLMISRTPEVTCVVVDVSHEDPEVKFNWYVDGVEVHNAKTKPREEQYNSTYRVVSVLTVLHQDWLNGKEYKCKVSNKALPAPIEKTISKAKGQPREPQVYTLPPSRDELTKNQVSLTCLVKGFYPSDIAVEWESNGQPENNYKTTPPVLDSDGSFFLYSKLTVDKSRWQQGNVFSCSVMHEALHNHYTQKSLSLSPGK

SEQ ID NO: 14 - protein, 237 aa, Artificial Sequence
  synthetic polypeptide
MGWSCIILFLVATATGVHSDIVLTQSPASLAVSLGQRATISCRASKSVSTSSYSYMHWYQQKPGQPPKLLIKYASYLESGVPARFSGSGSGTDFTLNIHPVEEEDAATYYCQHSREFPWTFGGGTKLEIKRTVAAPSVFIFPPSDEQLKSGTASVVCLLNNFYPREAKVQWKVDNALQSGNSQESVTEQDSKDSTYSLSSTLTLSKADYEKHKVYACEVTHQGLSSPVTKSFNRGEC

SEQ ID NO: 15 - protein, 5 aa, Artificial Sequence
  synthetic polypeptide
DYGMH

SEQ ID NO: 16 - protein, 5 aa, Artificial Sequence
  synthetic polypeptide
NYGMH

SEQ ID NO: 17 - protein, 17 aa, Artificial Sequence
  synthetic polypeptide
YISSGSSTIYYADTVKG

SEQ ID NO: 18 - protein, 7 aa, Artificial Sequence
  synthetic polypeptide
RGLLLDY

SEQ ID NO: 19 - protein, 17 aa, Artificial Sequence
  synthetic polypeptide
YISSGSSTIYYADSVKG

SEQ ID NO: 20 - protein, 8 aa, Artificial Sequence
  synthetic polypeptide
GFTFSDYG

SEQ ID NO: 21 - protein, 8 aa, Artificial Sequence
  synthetic polypeptide
GFTFSNYG

SEQ ID NO: 22 - protein, 8 aa, Artificial Sequence
  synthetic polypeptide
ISSGSSTI

SEQ ID NO: 23 - protein, 9 aa, Artificial Sequence
  synthetic polypeptide
ARRGLLLDY

SEQ ID NO: 24 - protein, 15 aa, Artificial Sequence
  synthetic polypeptide
RASKSVSTSSYSYMH

SEQ ID NO: 25 - protein, 7 aa, Artificial Sequence
  synthetic polypeptide
YASYLES

SEQ ID NO: 26 - protein, 9 aa, Artificial Sequence
  synthetic polypeptide
QHSREFPWT

SEQ ID NO: 27 - protein, 15 aa, Artificial Sequence
  synthetic polypeptide
RASKSVSTSSYSYLA

SEQ ID NO: 28 - protein, 7 aa, Artificial Sequence
  synthetic polypeptide
YASYLQS

SEQ ID NO: 29 - protein, 10 aa, Artificial Sequence
  synthetic polypeptide
KSVSTSSYSY

SEQ ID NO: 30 - protein, 3 aa, Artificial Sequence
  synthetic polypeptide
YAS

SEQ ID NO: 31 - protein, 7 aa, Artificial Sequence
  synthetic polypeptide
GQSSRSS

SEQ ID NO: 32 - protein, 18 aa, Artificial Sequence
  synthetic polypeptide
GQSSRSSSGGGSSGGGGS

SEQ ID NO: 33 - protein, 4 aa, Artificial Sequence
  synthetic polypeptide
GSGS

SEQ ID NO: 34 - protein, 4 aa, Artificial Sequence
  synthetic polypeptide
GGGS

SEQ ID NO: 35 - protein, 10 aa, Artificial Sequence
  synthetic polypeptide
GGGGSGGGGS

SEQ ID NO: 36 - protein, 20 aa, Artificial Sequence
  synthetic polypeptide
GGGGSGGGGSGGGGSGGGGS

SEQ ID NO: 37 - protein, 15 aa, Artificial Sequence
  synthetic polypeptide
GGGGSGGGGSGGGGS

SEQ ID NO: 38 - protein, 274 aa, Artificial Sequence
  synthetic polypeptide
AGIHDIVLTQSPASLAVSLGQRATISCRASKSVSTSSYSYMHWYQQKPGQPPKLLIKYASYLESGVPARFSGSGSGTDFTLNIHPVEEEDAATYYCQHSREFPWTFGGGTKLEIKRADAAPGGGGSGGGGSGGGGSEVQLVESGGGLVKPGGSRKLSCAASGFTFSNYGMHWVRQAPEKGLEWVAYISSGSSTIYYADTVKGRFTISRDNAKNTLFLQMTSLRSEDTAMYYCARRGLLLDYWGQGTTLTVSSLEQKLISEEDLNSAVDHHHHHH

SEQ ID NO: 39 - protein, 541 aa, Artificial Sequence
  synthetic polypeptide
AGIHDIVLTQSPASLAVSLGQRATISCRASKSVSTSSYSYMHWYQQKPGQPPKLLIKYASYLESGVPARFSGSGSGTDFTLNIHPVEEEDAATYYCQHSREFPWTFGGGTKLEIKRADAAPGGGGSGGGGSGGGGSEVQLVESGGGLVKPGGSRKLSCAASGFTFSNYGMHWVRQAPEKGLEWVAYISSGSSTIYYADTVKGRFTISRDNAKNTLFLQMTSLRSEDTAMYYCARRGLLLDYWGQGTTLTVSSASTKGPSVFPLAPLESSGSDIVLTQSPASLAVSLGQRATISCRASKSVSTSSYSYMHWYQQKPGQPPKLLIKYASYLESGVPARFSGSGSGTDFTLNIHPVEEEDAATYYCQHSREFPWTFGGGTKLEIKRADAAPGGGGSGGGGSGGGGSEVQLVESGGGLVKPGGSRKLSCAASGFTFSNYGMHWVRQAPEKGLEWVAYISSGSSTIYYADTVKGRFTISRDNAKNTLFLQMTSLRSEDTAMYYCARRGLLLDYWGQGTTLTVSSLEQKLISEEDLNSAVDHHHHHH

SEQ ID NO: 40 - protein, 808 aa, Artificial Sequence
  synthetic polypeptide
AGIHDIVLTQSPASLAVSLGQRATISCRASKSVSTSSYSYMHWYQQKPGQPPKLLIKYASYLESGVPARFSGSGSGTDFTLNIHPVEEEDAATYYCQHSREFPWTFGGGTKLEIKRADAAPGGGGSGGGGSGGGGSEVQLVESGGGLVKPGGSRKLSCAASGFTFSNYGMHWVRQAPEKGLEWVAYISSGSSTIYYADTVKGRFTISRDNAKNTLFLQMTSLRSEDTAMYYCARRGLLLDYWGQGTTLTVSSASTKGPSVFPLAPLESSGSDIVLTQSPASLAVSLGQRATISCRASKSVSTSSYSYMHWYQQKPGQPPKLLIKYASYLESGVPARFSGSGSGTDFTLNIHPVEEEDAATYYCQHSREFPWTFGGGTKLEIKRADAAPGGGGSGGGGSGGGGSEVQLVESGGGLVKPGGSRKLSCAASGFTFSNYGMHWVRQAPEKGLEWVAYISSGSSTIYYADTVKGRFTISRDNAKNTLFLQMTSLRSEDTAMYYCARRGLLLDYWGQGTTLTVSSASTKGPSVFPLAPLESSGSDIVLTQSPASLAVSLGQRATISCRASKSVSTSSYSYMHWYQQKPGQPPKLLIKYASYLESGVPARFSGSGSGTDFTLNIHPVEEEDAATYYCQHSREFPWTFGGGTKLEIKRADAAPGGGGSGGGGSGGGGSEVQLVESGGGLVKPGGSRKLSCAASGFTFSNYGMHWVRQAPEKGLEWVAYISSGSSTIYYADTVKGRFTISRDNAKNTLFLQMTSLRSEDTAMYYCARRGLLLDYWGQGTTLTVSSLEQKLISEEDLNSAVDHHHHHH

SEQ ID NO: 41 - protein, 242 aa, Artificial Sequence
  synthetic polypeptide
DIVLTQSPASLAVSPGQRATITCRASKSVSTSSYSYMHWYQQKPGQPPKLLIYYASYLESGVPARFSGSGSGTDFTLTINPVEANDTANYYCQHSREFPWTFGQGTKVEIKGGGGSGGGGSGGGGSEVQLVESGGGLVQPGGSLRLSCSASGFTFSNYGMHWVRQAPGKGLEYVSYISSGSSTIYYADTVKGRFTISRDNSKNTLYLQMSSLRAEDTAVYYCVKRGLLLDYWGQGTLVTVSS

SEQ ID NO: 42 - protein, 17 aa, Artificial Sequence
  synthetic polypeptide
YISSSSSTIYYADSVKG

SEQ ID NO: 43 - protein, 8 aa, Artificial Sequence
  synthetic polypeptide
ISSSSSTI

SEQ ID NO: 44 - protein, 15 aa, Artificial Sequence
  synthetic polypeptide
RASKTVSTSSYSYMH

SEQ ID NO: 45 - protein, 10 aa, Artificial Sequence
  synthetic polypeptide
KTVSTSSYSY

SEQ ID NO: 46 - protein, 116 aa, Artificial Sequence
  synthetic polypeptide
EVQLVESGGGLVQPGGSLRLSCAASGFTFSNYGMHWVRQAPGKGLEWVSYISSSSSTIYYADSVKGRFTISRDNAKNSLYLQMNSLRAEDTAVYYCARRGLLLDYWGQGTTVTVSS

SEQ ID NO: 47 - protein, 116 aa, Artificial Sequence
  synthetic polypeptide
EVQLVESGGGVVQPGGSLRLSCAASGFTFSNYGMHWVRQAPEKGLEWVSYISSSSSTIYYADSVKGRFTISRDNSKNTLYLQMNSLRAEDTAVYYCARRGLLLDYWGQGTTVTVSS

SEQ ID NO: 48 - protein, 116 aa, Artificial Sequence
  synthetic polypeptide
EVQLVESGGGDVKPGGSLRLSCAASGFTFSNYGMHWVRQAPEKGLEWVSYISSSSSTIYYADSVKGRFTISRDNSKNTLYLQMNSLRAEDTAVYYCARRGLLLDYWGQGTTVTVSS

SEQ ID NO: 49 - skipped
  synthetic polypeptide

SEQ ID NO: 50 - protein, 116 aa, Artificial Sequence
  synthetic polypeptide
EVQLVESGGGLVQPGGSLRLSCAASGFTFSNYGMHWVRQAPGKGLEWVSYISSGSSTIYYADSVKGRFTISRDNAKNSLYLQMNSLRAEDTAVYYCARRGLLLDYWGQGTTVTVSS

SEQ ID NO: 51 - protein, 116 aa, Artificial Sequence
  synthetic polypeptide
EVQLVESGGGVVQPGGSLRLSCAASGFTFSNYGMHWVRQAPEKGLEWVSYISSGSSTIYYADSVKGRFTISRDNSKNTLYLQMNSLRAEDTAVYYCARRGLLLDYWGQGTTVTVSS

SEQ ID NO: 52 - protein, 116 aa, Artificial Sequence
  synthetic polypeptide
EVQLVESGGGDVKPGGSLRLSCAASGFTFSNYGMHWVRQAPEKGLEWVSYISSGSSTIYYADSVKGRFTISRDNSKNTLYLQMNSLRAEDTAVYYCARRGLLLDYWGQGTTVTVSS

SEQ ID NO: 53 - protein, 111 aa, Artificial Sequence
  synthetic polypeptide
DIQMTQSPSSLSASLGDRATITCRASKSVSTSSYSYMHWYQQKPGQPPKLLIKYASYLESGVPSRFSGSGSGTDFTLTISSLQPEDAATYYCQHSREFPWTFGGGTKVEIK

SEQ ID NO: 54 - protein, 111 aa, Artificial Sequence
  synthetic polypeptide
DIQMTQSPSSLSASLGDRATITCRASKSVSTSSYSYMHWYQQKPGQAPKLLIKYASYLESGVPSRFSGSGSGTDFTLTISSLQPEDFATYYCQHSREFPWTFGQGTKVEIK

SEQ ID NO: 55 - protein, 111 aa, Artificial Sequence
  synthetic polypeptide
DIQMTQSPSSLSASVGDRVTITCRASKSVSTSSYSYMHWYQQKPGKAPKLLIKYASYLESGVPSRFSGSGSGTDFTLTISSLQPEDFATYYCQHSREFPWTFGQGTKVEIK

SEQ ID NO: 56 - protein, 111 aa, Artificial Sequence
  synthetic polypeptide
DIQMTQSPSSLSASLGDRATITCRASKTVSTSSYSYMHWYQQKPGQPPKLLIKYASYLESGVPSRFSGSGSGTDFTLTISSLQPEDAATYYCQHSREFPWTFGGGTKVEIK

SEQ ID NO: 57 - protein, 111 aa, Artificial Sequence
  synthetic polypeptide
DIQMTQSPSSLSASVGDRVTITCRASKTVSTSSYSYMHWYQQKPGKAPKLLIKYASYLESGVPSRFSGSGSGTDFTLTISSLQPEDFATYYCQHSREFPWTFGQGTKVEIK

SEQ ID NO: 58 - protein, 111 aa, Artificial Sequence
  synthetic polypeptide
DIQMTQSPSSLSASLGDRATITCRASKTVSTSSYSYMHWYQQKPGQAPKLLIKYASYLESGVPSRFSGSGSGTDFTLTISSLQPEDFATYYCQHSREFPWTFGQGTKVEIK

SEQ ID NO: 59 - protein, 21 aa, Artificial Sequence
  synthetic polypeptide
RADAAPGGGGSGGGGSGGGGS

SEQ ID NO: 60 - protein, 19 aa, Artificial Sequence
  synthetic polypeptide
ASTKGPSVFPLAPLESSGS

SEQ ID NO: 61 - protein, 515 aa, Artificial Sequence
  synthetic polypeptide
DIQMTQSPSSLSASLGDRATITCRASKSVSTSSYSYMHWYQQKPGQPPKLLIKYASYLESGVPSRFSGSGSGTDFTLTISSLQPEDAATYYCQHSREFPWTFGGGTKVEIKRADAAPGGGGSGGGGSGGGGSEVQLVESGGGLVQPGGSLRLSCAASGFTFSNYGMHWVRQAPGKGLEWVSYISSSSSTIYYADSVKGRFTISRDNAKNSLYLQMNSLRAEDTAVYYCARRGLLLDYWGQGTTVTVSSASTKGPSVFPLAPLESSGSDIQMTQSPSSLSASLGDRATITCRASKSVSTSSYSYMHWYQQKPGQPPKLLIKYASYLESGVPSRFSGSGSGTDFTLTISSLQPEDAATYYCQHSREFPWTFGGGTKVEIKRADAAPGGGGSGGGGSGGGGSEVQLVESGGGLVQPGGSLRLSCAASGFTFSNYGMHWVRQAPGKGLEWVSYISSSSSTIYYADSVKGRFTISRDNAKNSLYLQMNSLRAEDTAVYYCARRGLLLDYWGQGTTVTVSS

SEQ ID NO: 62 - protein, 515 aa, Artificial Sequence
  synthetic polypeptide
DIQMTQSPSSLSASLGDRATITCRASKSVSTSSYSYMHWYQQKPGQPPKLLIKYASYLESGVPSRFSGSGSGTDFTLTISSLQPEDAATYYCQHSREFPWTFGGGTKVEIKRADAAPGGGGSGGGGSGGGGSEVQLVESGGGVVQPGGSLRLSCAASGFTFSNYGMHWVRQAPEKGLEWVSYISSSSSTIYYADSVKGRFTISRDNSKNTLYLQMNSLRAEDTAVYYCARRGLLLDYWGQGTTVTVSSASTKGPSVFPLAPLESSGSDIQMTQSPSSLSASLGDRATITCRASKSVSTSSYSYMHWYQQKPGQPPKLLIKYASYLESGVPSRFSGSGSGTDFTLTISSLQPEDAATYYCQHSREFPWTFGGGTKVEIKRADAAPGGGGSGGGGSGGGGSEVQLVESGGGVVQPGGSLRLSCAASGFTFSNYGMHWVRQAPEKGLEWVSYISSSSSTIYYADSVKGRFTISRDNSKNTLYLQMNSLRAEDTAVYYCARRGLLLDYWGQGTTVTVSS

SEQ ID NO: 63 - protein, 515 aa, Artificial Sequence
  synthetic polypeptide
DIQMTQSPSSLSASLGDRATITCRASKSVSTSSYSYMHWYQQKPGQPPKLLIKYASYLESGVPSRFSGSGSGTDFTLTISSLQPEDAATYYCQHSREFPWTFGGGTKVEIKRADAAPGGGGSGGGGSGGGGSEVQLVESGGGDVKPGGSLRLSCAASGFTFSNYGMHWVRQAPEKGLEWVSYISSSSSTIYYADSVKGRFTISRDNSKNTLYLQMNSLRAEDTAVYYCARRGLLLDYWGQGTTVTVSSASTKGPSVFPLAPLESSGSDIQMTQSPSSLSASLGDRATITCRASKSVSTSSYSYMHWYQQKPGQPPKLLIKYASYLESGVPSRFSGSGSGTDFTLTISSLQPEDAATYYCQHSREFPWTFGGGTKVEIKRADAAPGGGGSGGGGSGGGGSEVQLVESGGGDVKPGGSLRLSCAASGFTFSNYGMHWVRQAPEKGLEWVSYISSSSSTIYYADSVKGRFTISRDNSKNTLYLQMNSLRAEDTAVYYCARRGLLLDYWGQGTTVTVSS

SEQ ID NO: 64 - protein, 515 aa, Artificial Sequence
  synthetic polypeptide
DIQMTQSPSSLSASLGDRATITCRASKSVSTSSYSYMHWYQQKPGQAPKLLIKYASYLESGVPSRFSGSGSGTDFTLTISSLQPEDFATYYCQHSREFPWTFGQGTKVEIKRADAAPGGGGSGGGGSGGGGSEVQLVESGGGLVQPGGSLRLSCAASGFTFSNYGMHWVRQAPGKGLEWVSYISSSSSTIYYADSVKGRFTISRDNAKNSLYLQMNSLRAEDTAVYYCARRGLLLDYWGQGTTVTVSSASTKGPSVFPLAPLESSGSDIQMTQSPSSLSASLGDRATITCRASKSVSTSSYSYMHWYQQKPGQAPKLLIKYASYLESGVPSRFSGSGSGTDFTLTISSLQPEDFATYYCQHSREFPWTFGQGTKVEIKRADAAPGGGGSGGGGSGGGGSEVQLVESGGGLVQPGGSLRLSCAASGFTFSNYGMHWVRQAPGKGLEWVSYISSSSSTIYYADSVKGRFTISRDNAKNSLYLQMNSLRAEDTAVYYCARRGLLLDYWGQGTTVTVSS

SEQ ID NO: 65 - protein, 515 aa, Artificial Sequence
  synthetic polypeptide
DIQMTQSPSSLSASLGDRATITCRASKSVSTSSYSYMHWYQQKPGQAPKLLIKYASYLESGVPSRFSGSGSGTDFTLTISSLQPEDFATYYCQHSREFPWTFGQGTKVEIKRADAAPGGGGSGGGGSGGGGSEVQLVESGGGVVQPGGSLRLSCAASGFTFSNYGMHWVRQAPEKGLEWVSYISSSSSTIYYADSVKGRFTISRDNSKNTLYLQMNSLRAEDTAVYYCARRGLLLDYWGQGTTVTVSSASTKGPSVFPLAPLESSGSDIQMTQSPSSLSASLGDRATITCRASKSVSTSSYSYMHWYQQKPGQAPKLLIKYASYLESGVPSRFSGSGSGTDFTLTISSLQPEDFATYYCQHSREFPWTFGQGTKVEIKRADAAPGGGGSGGGGSGGGGSEVQLVESGGGVVQPGGSLRLSCAASGFTFSNYGMHWVRQAPEKGLEWVSYISSSSSTIYYADSVKGRFTISRDNSKNTLYLQMNSLRAEDTAVYYCARRGLLLDYWGQGTTVTVSS

SEQ ID NO: 66 - protein, 515 aa, Artificial Sequence
  synthetic polypeptide
DIQMTQSPSSLSASLGDRATITCRASKSVSTSSYSYMHWYQQKPGQAPKLLIKYASYLESGVPSRFSGSGSGTDFTLTISSLQPEDFATYYCQHSREFPWTFGQGTKVEIKRADAAPGGGGSGGGGSGGGGSEVQLVESGGGDVKPGGSLRLSCAASGFTFSNYGMHWVRQAPEKGLEWVSYISSSSSTIYYADSVKGRFTISRDNSKNTLYLQMNSLRAEDTAVYYCARRGLLLDYWGQGTTVTVSSASTKGPSVFPLAPLESSGSDIQMTQSPSSLSASLGDRATITCRASKSVSTSSYSYMHWYQQKPGQAPKLLIKYASYLESGVPSRFSGSGSGTDFTLTISSLQPEDFATYYCQHSREFPWTFGQGTKVEIKRADAAPGGGGSGGGGSGGGGSEVQLVESGGGDVKPGGSLRLSCAASGFTFSNYGMHWVRQAPEKGLEWVSYISSSSSTIYYADSVKGRFTISRDNSKNTLYLQMNSLRAEDTAVYYCARRGLLLDYWGQGTTVTVSS

SEQ ID NO: 67 - protein, 515 aa, Artificial Sequence
  synthetic polypeptide
DIQMTQSPSSLSASVGDRVTITCRASKSVSTSSYSYMHWYQQKPGKAPKLLIKYASYLESGVPSRFSGSGSGTDFTLTISSLQPEDFATYYCQHSREFPWTFGQGTKVEIKRADAAPGGGGSGGGGSGGGGSEVQLVESGGGLVQPGGSLRLSCAASGFTFSNYGMHWVRQAPGKGLEWVSYISSSSSTIYYADSVKGRFTISRDNAKNSLYLQMNSLRAEDTAVYYCARRGLLLDYWGQGTTVTVSSASTKGPSVFPLAPLESSGSDIQMTQSPSSLSASVGDRVTITCRASKSVSTSSYSYMHWYQQKPGKAPKLLIKYASYLESGVPSRFSGSGSGTDFTLTISSLQPEDFATYYCQHSREFPWTFGQGTKVEIKRADAAPGGGGSGGGGSGGGGSEVQLVESGGGLVQPGGSLRLSCAASGFTFSNYGMHWVRQAPGKGLEWVSYISSSSSTIYYADSVKGRFTISRDNAKNSLYLQMNSLRAEDTAVYYCARRGLLLDYWGQGTTVTVSS

SEQ ID NO: 68 - protein, 515 aa, Artificial Sequence
  synthetic polypeptide
DIQMTQSPSSLSASVGDRVTITCRASKSVSTSSYSYMHWYQQKPGKAPKLLIKYASYLESGVPSRFSGSGSGTDFTLTISSLQPEDFATYYCQHSREFPWTFGQGTKVEIKRADAAPGGGGSGGGGSGGGGSEVQLVESGGGVVQPGGSLRLSCAASGFTFSNYGMHWVRQAPEKGLEWVSYISSSSSTIYYADSVKGRFTISRDNSKNTLYLQMNSLRAEDTAVYYCARRGLLLDYWGQGTTVTVSSASTKGPSVFPLAPLESSGSDIQMTQSPSSLSASVGDRVTITCRASKSVSTSSYSYMHWYQQKPGKAPKLLIKYASYLESGVPSRFSGSGSGTDFTLTISSLQPEDFATYYCQHSREFPWTFGQGTKVEIKRADAAPGGGGSGGGGSGGGGSEVQLVESGGGVVQPGGSLRLSCAASGFTFSNYGMHWVRQAPEKGLEWVSYISSSSSTIYYADSVKGRFTISRDNSKNTLYLQMNSLRAEDTAVYYCARRGLLLDYWGQGTTVTVSS

SEQ ID NO: 69 - protein, 515 aa, Artificial Sequence
  synthetic polypeptide
DIQMTQSPSSLSASVGDRVTITCRASKSVSTSSYSYMHWYQQKPGKAPKLLIKYASYLESGVPSRFSGSGSGTDFTLTISSLQPEDFATYYCQHSREFPWTFGQGTKVEIKRADAAPGGGGSGGGGSGGGGSEVQLVESGGGDVKPGGSLRLSCAASGFTFSNYGMHWVRQAPEKGLEWVSYISSSSSTIYYADSVKGRFTISRDNSKNTLYLQMNSLRAEDTAVYYCARRGLLLDYWGQGTTVTVSSASTKGPSVFPLAPLESSGSDIQMTQSPSSLSASVGDRVTITCRASKSVSTSSYSYMHWYQQKPGKAPKLLIKYASYLESGVPSRFSGSGSGTDFTLTISSLQPEDFATYYCQHSREFPWTFGQGTKVEIKRADAAPGGGGSGGGGSGGGGSEVQLVESGGGDVKPGGSLRLSCAASGFTFSNYGMHWVRQAPEKGLEWVSYISSSSSTIYYADSVKGRFTISRDNSKNTLYLQMNSLRAEDTAVYYCARRGLLLDYWGQGTTVTVSS

SEQ ID NO: 70 - protein, 515 aa, Artificial Sequence
  synthetic polypeptide
DIQMTQSPSSLSASLGDRATITCRASKTVSTSSYSYMHWYQQKPGQPPKLLIKYASYLESGVPSRFSGSGSGTDFTLTISSLQPEDAATYYCQHSREFPWTFGGGTKVEIKRADAAPGGGGSGGGGSGGGGSEVQLVESGGGLVQPGGSLRLSCAASGFTFSNYGMHWVRQAPGKGLEWVSYISSGSSTIYYADSVKGRFTISRDNAKNSLYLQMNSLRAEDTAVYYCARRGLLLDYWGQGTTVTVSSASTKGPSVFPLAPLESSGSDIQMTQSPSSLSASLGDRATITCRASKTVSTSSYSYMHWYQQKPGQPPKLLIKYASYLESGVPSRFSGSGSGTDFTLTISSLQPEDAATYYCQHSREFPWTFGGGTKVEIKRADAAPGGGGSGGGGSGGGGSEVQLVESGGGLVQPGGSLRLSCAASGFTFSNYGMHWVRQAPGKGLEWVSYISSGSSTIYYADSVKGRFTISRDNAKNSLYLQMNSLRAEDTAVYYCARRGLLLDYWGQGTTVTVSS

SEQ ID NO: 71 - protein, 515 aa, Artificial Sequence
  synthetic polypeptide
DIQMTQSPSSLSASLGDRATITCRASKTVSTSSYSYMHWYQQKPGQPPKLLIKYASYLESGVPSRFSGSGSGTDFTLTISSLQPEDAATYYCQHSREFPWTFGGGTKVEIKRADAAPGGGGSGGGGSGGGGSEVQLVESGGGVVQPGGSLRLSCAASGFTFSNYGMHWVRQAPEKGLEWVSYISSGSSTIYYADSVKGRFTISRDNSKNTLYLQMNSLRAEDTAVYYCARRGLLLDYWGQGTTVTVSSASTKGPSVFPLAPLESSGSDIQMTQSPSSLSASLGDRATITCRASKTVSTSSYSYMHWYQQKPGQPPKLLIKYASYLESGVPSRFSGSGSGTDFTLTISSLQPEDAATYYCQHSREFPWTFGGGTKVEIKRADAAPGGGGSGGGGSGGGGSEVQLVESGGGVVQPGGSLRLSCAASGFTFSNYGMHWVRQAPEKGLEWVSYISSGSSTIYYADSVKGRFTISRDNSKNTLYLQMNSLRAEDTAVYYCARRGLLLDYWGQGTTVTVSS

SEQ ID NO: 72 - protein, 515 aa, Artificial Sequence
  synthetic polypeptide
DIQMTQSPSSLSASLGDRATITCRASKTVSTSSYSYMHWYQQKPGQPPKLLIKYASYLESGVPSRFSGSGSGTDFTLTISSLQPEDAATYYCQHSREFPWTFGGGTKVEIKRADAAPGGGGSGGGGSGGGGSEVQLVESGGGDVKPGGSLRLSCAASGFTFSNYGMHWVRQAPEKGLEWVSYISSGSSTIYYADSVKGRFTISRDNSKNTLYLQMNSLRAEDTAVYYCARRGLLLDYWGQGTTVTVSSASTKGPSVFPLAPLESSGSDIQMTQSPSSLSASLGDRATITCRASKTVSTSSYSYMHWYQQKPGQPPKLLIKYASYLESGVPSRFSGSGSGTDFTLTISSLQPEDAATYYCQHSREFPWTFGGGTKVEIKRADAAPGGGGSGGGGSGGGGSEVQLVESGGGDVKPGGSLRLSCAASGFTFSNYGMHWVRQAPEKGLEWVSYISSGSSTIYYADSVKGRFTISRDNSKNTLYLQMNSLRAEDTAVYYCARRGLLLDYWGQGTTVTVSS

SEQ ID NO: 73 - protein, 515 aa, Artificial Sequence
  synthetic polypeptide
DIQMTQSPSSLSASVGDRVTITCRASKTVSTSSYSYMHWYQQKPGKAPKLLIKYASYLESGVPSRFSGSGSGTDFTLTISSLQPEDFATYYCQHSREFPWTFGQGTKVEIKRADAAPGGGGSGGGGSGGGGSEVQLVESGGGLVQPGGSLRLSCAASGFTFSNYGMHWVRQAPGKGLEWVSYISSGSSTIYYADSVKGRFTISRDNAKNSLYLQMNSLRAEDTAVYYCARRGLLLDYWGQGTTVTVSSASTKGPSVFPLAPLESSGSDIQMTQSPSSLSASVGDRVTITCRASKTVSTSSYSYMHWYQQKPGKAPKLLIKYASYLESGVPSRFSGSGSGTDFTLTISSLQPEDFATYYCQHSREFPWTFGQGTKVEIKRADAAPGGGGSGGGGSGGGGSEVQLVESGGGLVQPGGSLRLSCAASGFTFSNYGMHWVRQAPGKGLEWVSYISSGSSTIYYADSVKGRFTISRDNAKNSLYLQMNSLRAEDTAVYYCARRGLLLDYWGQGTTVTVSS

SEQ ID NO: 74 - protein, 515 aa, Artificial Sequence
  synthetic polypeptide
DIQMTQSPSSLSASVGDRVTITCRASKTVSTSSYSYMHWYQQKPGKAPKLLIKYASYLESGVPSRFSGSGSGTDFTLTISSLQPEDFATYYCQHSREFPWTFGQGTKVEIKRADAAPGGGGSGGGGSGGGGSEVQLVESGGGVVQPGGSLRLSCAASGFTFSNYGMHWVRQAPEKGLEWVSYISSGSSTIYYADSVKGRFTISRDNSKNTLYLQMNSLRAEDTAVYYCARRGLLLDYWGQGTTVTVSSASTKGPSVFPLAPLESSGSDIQMTQSPSSLSASVGDRVTITCRASKTVSTSSYSYMHWYQQKPGKAPKLLIKYASYLESGVPSRFSGSGSGTDFTLTISSLQPEDFATYYCQHSREFPWTFGQGTKVEIKRADAAPGGGGSGGGGSGGGGSEVQLVESGGGVVQPGGSLRLSCAASGFTFSNYGMHWVRQAPEKGLEWVSYISSGSSTIYYADSVKGRFTISRDNSKNTLYLQMNSLRAEDTAVYYCARRGLLLDYWGQGTTVTVSS

SEQ ID NO: 75 - protein, 515 aa, Artificial Sequence
  synthetic polypeptide
DIQMTQSPSSLSASVGDRVTITCRASKTVSTSSYSYMHWYQQKPGKAPKLLIKYASYLESGVPSRFSGSGSGTDFTLTISSLQPEDFATYYCQHSREFPWTFGQGTKVEIKRADAAPGGGGSGGGGSGGGGSEVQLVESGGGDVKPGGSLRLSCAASGFTFSNYGMHWVRQAPEKGLEWVSYISSGSSTIYYADSVKGRFTISRDNSKNTLYLQMNSLRAEDTAVYYCARRGLLLDYWGQGTTVTVSSASTKGPSVFPLAPLESSGSDIQMTQSPSSLSASVGDRVTITCRASKTVSTSSYSYMHWYQQKPGKAPKLLIKYASYLESGVPSRFSGSGSGTDFTLTISSLQPEDFATYYCQHSREFPWTFGQGTKVEIKRADAAPGGGGSGGGGSGGGGSEVQLVESGGGDVKPGGSLRLSCAASGFTFSNYGMHWVRQAPEKGLEWVSYISSGSSTIYYADSVKGRFTISRDNSKNTLYLQMNSLRAEDTAVYYCARRGLLLDYWGQGTTVTVSS

SEQ ID NO: 76 - protein, 515 aa, Artificial Sequence
  synthetic polypeptide
DIQMTQSPSSLSASLGDRATITCRASKTVSTSSYSYMHWYQQKPGQAPKLLIKYASYLESGVPSRFSGSGSGTDFTLTISSLQPEDFATYYCQHSREFPWTFGQGTKVEIKRADAAPGGGGSGGGGSGGGGSEVQLVESGGGLVQPGGSLRLSCAASGFTFSNYGMHWVRQAPGKGLEWVSYISSGSSTIYYADSVKGRFTISRDNAKNSLYLQMNSLRAEDTAVYYCARRGLLLDYWGQGTTVTVSSASTKGPSVFPLAPLESSGSDIQMTQSPSSLSASLGDRATITCRASKTVSTSSYSYMHWYQQKPGQAPKLLIKYASYLESGVPSRFSGSGSGTDFTLTISSLQPEDFATYYCQHSREFPWTFGQGTKVEIKRADAAPGGGGSGGGGSGGGGSEVQLVESGGGLVQPGGSLRLSCAASGFTFSNYGMHWVRQAPGKGLEWVSYISSGSSTIYYADSVKGRFTISRDNAKNSLYLQMNSLRAEDTAVYYCARRGLLLDYWGQGTTVTVSS

SEQ ID NO: 77 - protein, 446 aa, Artificial Sequence
  synthetic polypeptide
EVQLVESGGGLVQPGGSLRLSCAASGFTFSNYGMHWVRQAPGKGLEWVSYISSGSSTIYYADSVKGRFTISRDNAKNSLYLQMNSLRAEDTAVYYCARRGLLLDYWGQGTTVTVSSASTKGPSVFPLAPSSKSTSGGTAALGCLVKDYFPEPVTVSWNSGALTSGVHTFPAVLQSSGLYSLSSVVTVPSSSLGTQTYICNVNHKPSNTKVDKKVEPKSCDKTHTCPPCPAPEAAGGPSVFLFPPKPKDTLMISRTPEVTCVVVDVSHEDPEVKFNWYVDGVEVHNAKTKPREEQYNSTYRVVSVLTVLHQDWLNGKEYKCKVSNKALPAPIEKTISKAKGQPREPQVYTLPPSRDELTKNQVSLTCLVKGFYPSDIAVEWESNGQPENNYKTTPPVLDSDGSFFLYSKLTVDKSRWQQGNVFSCSVMHEALHNHYTQKSLSLSPGK

SEQ ID NO: 78 - protein, 98 aa, Artificial Sequence
  synthetic polypeptide
ASTKGPSVFPLAPSSKSTSGGTAALGCLVKDYFPEPVTVSWNSGALTSGVHTFPAVLQSSGLYSLSSVVTVPSSSLGTQTYICNVNHKPSNTKVDKKV

SEQ ID NO: 79 - protein, 12 aa, Artificial Sequence
  synthetic polypeptide
EPKSCDKTHTCP

SEQ ID NO: 80 - protein, 113 aa, Artificial Sequence
  synthetic polypeptide
PCPAPEAAGGPSVFLFPPKPKDTLMISRTPEVTCVVVDVSHEDPEVKFNWYVDGVEVHNAKTKPREEQYNSTYRVVSVLTVLHQDWLNGKEYKCKVSNKALPAPIEKTISKAK

SEQ ID NO: 81 - protein, 107 aa, Artificial Sequence
  synthetic polypeptide
GQPREPQVYTLPPSRDELTKNQVSLTCLVKGFYPSDIAVEWESNGQPENNYKTTPPVLDSDGSFFLYSKLTVDKSRWQQGNVFSCSVMHEALHNHYTQKSLSLSPGK

SEQ ID NO: 82 - protein, 446 aa, Artificial Sequence
  synthetic polypeptide
EVQLVESGGGLVQPGGSLRLSCAASGFTFSNYGMHWVRQAPGKGLEWVSYISSGSSTIYYADSVKGRFTISRDNAKNSLYLQMNSLRAEDTAVYYCARRGLLLDYWGQGTTVTVSSASTKGPSVFPLAPSSKSTSGGTAALGCLVKDYFPEPVTVSWNSGALTSGVHTFPAVLQSSGLYSLSSVVTVPSSSLGTQTYICNVNHKPSNTKVDKKVEPKSCDKTHTCPPCPAPELLGGPSVFLFPPKPKDTLMISRTPEVTCVVVDVSHEDPEVKFNWYVDGVEVHNAKTKPREEQYDSTYRVVSVLTVLHQDWLNGKEYKCKVSNKALPAPIEKTISKAKGQPREPQVYTLPPSRDELTKNQVSLTCLVKGFYPSDIAVEWESNGQPENNYKTTPPVLDSDGSFFLYSKLTVDKSRWQQGNVFSCSVMHEALHNHYTQKSLSLSPGK

SEQ ID NO: 83 - protein, 113 aa, Artificial Sequence
  synthetic polypeptide
PCPAPELLGGPSVFLFPPKPKDTLMISRTPEVTCVVVDVSHEDPEVKFNWYVDGVEVHNAKTKPREEQYDSTYRVVSVLTVLHQDWLNGKEYKCKVSNKALPAPIEKTISKAK

SEQ ID NO: 84 - protein, 446 aa, Artificial Sequence
  synthetic polypeptide
EVQLVESGGGLVQPGGSLRLSCAASGFTFSNYGMHWVRQAPGKGLEWVSYISSGSSTIYYADSVKGRFTISRDNAKNSLYLQMNSLRAEDTAVYYCARRGLLLDYWGQGTTVTVSSASTKGPSVFPLAPSSKSTSGGTAALGCLVKDYFPEPVTVSWNSGALTSGVHTFPAVLQSSGLYSLSSVVTVPSSSLGTQTYICNVNHKPSNTKVDKKVEPKSCDKTHTCPPCPAPEAAGGPSVFLFPPKPKDTLMISRTPEVTCVVVDVSHEDPEVKFNWYVDGVEVHNAKTKPREEQYDSTYRVVSVLTVLHQDWLNGKEYKCKVSNKALPAPIEKTISKAKGQPREPQVYTLPPSRDELTKNQVSLTCLVKGFYPSDIAVEWESNGQPENNYKTTPPVLDSDGSFFLYSKLTVDKSRWQQGNVFSCSVMHEALHNHYTQKSLSLSPGK

SEQ ID NO: 85 - protein, 113 aa, Artificial Sequence
  synthetic polypeptide
PCPAPEAAGGPSVFLFPPKPKDTLMISRTPEVTCVVVDVSHEDPEVKFNWYVDGVEVHNAKTKPREEQYDSTYRVVSVLTVLHQDWLNGKEYKCKVSNKALPAPIEKTISKAK

SEQ ID NO: 86 - protein, 113 aa, Artificial Sequence
  synthetic polypeptide
PCPAPELLGGPSVFLFPPKPKDTLMISRTPEVTCVVVDVSHEDPEVKFNWYVDGVEVHNAKTKPREEQYNSTYRVVSVLTVLHQDWLNGKEYKCKVSNKALPAPIEKTISKAK

SEQ ID NO: 87 - protein, 218 aa, Artificial Sequence
  synthetic polypeptide
DIQMTQSPSSLSASLGDRATITCRASKTVSTSSYSYMHWYQQKPGQPPKLLIKYASYLESGVPSRFSGSGSGTDFTLTISSLQPEDAATYYCQHSREFPWTFGGGTKLEIKRTVAAPSVFIFPPSDEQLKSGTASVVCLLNNFYPREAKVQWKVDNALQSGNSQESVTEQDSKDSTYSLSSTLTLSKADYEKHKVYACEVTHQGLSSPVTKSFNRGEC

SEQ ID NO: 88 - protein, 31 aa, Artificial Sequence
  synthetic polypeptide
RASKSVSTSSYSYMHWYQQKPGQPPKLLIKY

SEQ ID NO: 89 - protein, 31 aa, Artificial Sequence
  synthetic polypeptide
RASKTVSTSSYSYMHWYQQKPGQPPKLLIKY

SEQ ID NO: 90 - protein, 33 aa, Artificial Sequence
  synthetic polypeptide
RVTITCRASKSVSTSSYSYMHWYQQKPGKAPKL

SEQ ID NO: 91 - protein, 32 aa, Artificial Sequence
  synthetic polypeptide
  MISC_FEATURE (1)..(1): X = any amino acid, but preferentially is a basic residue (R or K)
  MISC_FEATURE (30)..(30): X = any amino acid, but preferentially is a basic residue (R or K)
XRASKTVSTSSYSYMHWYQQKPGQPPKLLXKY

SEQ ID NO: 92 - protein, 115 aa, Artificial Sequence
  synthetic polypeptide
EVQLVESGGGLVKPGGSRKLSCAASGFTFSDYGMHWVRQAPEKGLEWVAYISSGSSTIYYADTVKGRFTISRDNAKNTLFLQMTSLRSEDTAMYYCARRGLLLDYWGQGTTLTVS

SEQ ID NO: 93 - protein, 132 aa, Artificial Sequence
  synthetic polypeptide
DIVLTQSPASLAVSLGQRATISCRASKSVSTSSYSYMHWYQQKPGQPPKLLIKYASYLESGVPARFSGSGSGTDFTLNIHPVEEEDAATYYCQHSREFPWTFGGGTKLEIKRADAAPGGGGSGGGGSGGGGS